European Patent Application EP 4 147 696 A1, published March 15, 2023. Title: CHIMERIC PROTEIN. Applicant: Autolus Limited. The sequence listing filed with the application follows.

SEQUENCE LISTING (17 sequences)

SEQ ID NO: 1 - protein, 517 aa, synthetic construct
  REGION 1..517: note = Chimeric protein FRB-FKBP12-L3-dCasp9
MASRILWHEMWHEGLEEASRLYFGERNVKGMFEVLEPLHAMMERGPQTLKETSFNQAYGRDLMEAQEWCRKYMKSGNVKDLLQAWDLYYHVFRRISKLEYSGGGSLEGVQVETISPGDGRTFPKRGQTCVVHYTGMLEDGKKFDSSRDRNKPFKFMLGKQEVIRGWEEGVAQMSVGQRAKLTISPDYAYGATGHPGIIPPHATLVFDVELLKLESGGGGSGGGGSGGGGSGVDGFGDVGALESLRGNADLAYILSMEPCGHCLIINNVNFCRESGLRTRTGSNIDCEKLRRRFSSLHFMVEVKGDLTAKKMVLALLELAQQDHGALDCCVVVILSHGCQASHLQFPGAVYGTDGCPVSVEKIVNIFNGTSCPSLGGKPKLFFIQACGGEQKDHGFEVASTSPEDESPGSNPEPDATPFQEGLRTFDQLDAISSLPTPSDIFVSYSTFPGFVSWRDPKSGSWYVETLDDIFEQWAHSEDLQSLLLRVANAVSVKGIYKQMPGCFNFLRKKLFFKTSAS

SEQ ID NO: 2 - protein, 402 aa, synthetic construct
  REGION 1..402: note = Chimeric protein FKBP12-dCasp9
MLEGVQVETISPGDGRTFPKRGQTCVVHYTGMLEDGKKFDSSRDRNKPFKFMLGKQEVIRGWEEGVAQMSVGQRAKLTISPDYAYGATGHPGIIPPHATLVFDVELLKLESGGGSGVDGFGDVGALESLRGNADLAYILSMEPCGHCLIINNVNFCRESGLRTRTGSNIDCEKLRRRFSSLHFMVEVKGDLTAKKMVLALLELAQQDHGALDCCVVVILSHGCQASHLQFPGAVYGTDGCPVSVEKIVNIFNGTSCPSLGGKPKLFFIQACGGEQKDHGFEVASTSPEDESPGSNPEPDATPFQEGLRTFDQLDAISSLPTPSDIFVSYSTFPGFVSWRDPKSGSWYVETLDDIFEQWAHSEDLQSLLLRVANAVSVKGIYKQMPGCFNFLRKKLFFKTSAS

SEQ ID NO: 3 - protein, 392 aa, synthetic construct
  REGION 1..392: note = Chimeric protein FRB-dCasp9
MASRILWHEMWHEGLEEASRLYFGERNVKGMFEVLEPLHAMMERGPQTLKETSFNQAYGRDLMEAQEWCRKYMKSGNVKDLLQAWDLYYHVFRRISKLEYSGGGSGVDGFGDVGALESLRGNADLAYILSMEPCGHCLIINNVNFCRESGLRTRTGSNIDCEKLRRRFSSLHFMVEVKGDLTAKKMVLALLELAQQDHGALDCCVVVILSHGCQASHLQFPGAVYGTDGCPVSVEKIVNIFNGTSCPSLGGKPKLFFIQACGGEQKDHGFEVASTSPEDESPGSNPEPDATPFQEGLRTFDQLDAISSLPTPSDIFVSYSTFPGFVSWRDPKSGSWYVETLDDIFEQWAHSEDLQSLLLRVANAVSVKGIYKQMPGCFNFLRKKLFFKTSAS

SEQ ID NO: 4 - protein, 651 aa, synthetic construct
  REGION 1..651: note = Chimeric protein FKBP12-dCasp9-2A-FRB-FRBw
MLEGVQVETISPGDGRTFPKRGQTCVVHYTGMLEDGKKFDSSRDRNKPFKFMLGKQEVIRGWEEGVAQMSVGQRAKLTISPDYAYGATGHPGIIPPHATLVFDVELLKLESGGGSGVDGFGDVGALESLRGNADLAYILSMEPCGHCLIINNVNFCRESGLRTRTGSNIDCEKLRRRFSSLHFMVEVKGDLTAKKMVLALLELAQQDHGALDCCVVVILSHGCQASHLQFPGAVYGTDGCPVSVEKIVNIFNGTSCPSLGGKPKLFFIQACGGEQKDHGFEVASTSPEDESPGSNPEPDATPFQEGLRTFDQLDAISSLPTPSDIFVSYSTFPGFVSWRDPKSGSWYVETLDDIFEQWAHSEDLQSLLLRVANAVSVKGIYKQMPGCFNFLRKKLFFKTSASQCTNYALLKLAGDVESNPGPGVQVETISPGDGRTFPKRGQTCVVHYTGMLEDGKKVDSSRDRNKPFKFMLGKQEVIRGWEEGVAQMSVGQRAKLTISPDYAYGATGHPGIIPPHATLVFDVELLKLESGGGGSGGGGSMLEGVQVETISPGDGRTFPKRGQTCVVHYTGMLEDGKKFDSSRDRNKPFKFMLGKQEVIRGWEEGVAQMSVGQRAKLTISPDYAYGATGHPGIIPPHATLVFDVELLKLES

SEQ ID NO: 5 - protein, 416 aa, Homo sapiens [sequence omitted]

SEQ ID NO: 6 - protein, 282 aa, Homo sapiens
GFGDVGALESLRGNADLAYILSMEPCGHCLIINNVNFCRESGLRTRTGSNIDCEKLRRRFSSLHFMVEVKGDLTAKKMVLALLELAQQDHGALDCCVVVILSHGCQASHLQFPGAVYGTDGCPVSVEKIVNIFNGTSCPSLGGKPKLFFIQACGGEQKDHGFEVASTSPEDESPGSNPEPDATPFQEGLRTFDQLDAISSLPTPSDIFVSYSTFPGFVSWRDPKSGSWYVETLDDIFEQWAHSEDLQSLLLRVANAVSVKGIYKQMPGCFNFLRKKLFFKTS

SEQ ID NO: 7 - protein, 108 aa, synthetic construct
  REGION 1..108: note = FKBP12 domain
MGVQVETISPGDGRTFPKRGQTCVVHYTGMLEDGKKFDSSRDRNKPFKFMLGKQEVIRGWEEGVAQMSVGQRAKLTISPDYAYGATGHPGIIPPHATLVFDVELLKLE

SEQ ID NO: 8 - protein, 100 aa, synthetic construct
  REGION 1..100: note = wild-type FRB segment of mTOR
MASRILWHEMWHEGLEEASRLYFGERNVKGMFEVLEPLHAMMERGPQTLKETSFNQAYGRDLMEAQEWCRKYMKSGNVKDLTQAWDLYYHVFRRISKLES

SEQ ID NO: 9 - protein, 100 aa, synthetic construct
  REGION 1..100: note = FRB with T to L substitution at 2098 which allows binding toAP21967
MASRILWHEMWHEGLEEASRLYFGERNVKGMFEVLEPLHAMMERGPQTLKETSFNQAYGRDLMEAQEWCRKYMKSGNVKDLLQAWDLYYHVFRRISKLES

SEQ ID NO: 10 - protein, 100 aa, synthetic construct
  REGION 1..100: note = FRB segment of mTOR with T to H substitution at 2098 and to W atF at residue 2101 of the full mTOR
MASRILWHEMWHEGLEEASRLYFGERNVKGMFEVLEPLHAMMERGPQTLKETSFNQAYGRDLMEAQEWCRKYMKSGNVKDLHQAFDLYYHVFRRISKLES

SEQ ID NO: 11 - protein, 100 aa, synthetic construct
  REGION 1..100: note = FRB segment of mTOR with K to P substitution at residue 2095 ofthe full mTOR
MASRILWHEMWHEGLEEASRLYFGERNVKGMFEVLEPLHAMMERGPQTLKETSFNQAYGRDLMEAQEWCRKYMKSGNVPDLTQAWDLYYHVFRRISKLES

SEQ ID NO: 12 - DNA, 1554 bp, synthetic construct
  misc_feature 1..1554: note = FRB-FKBP12-L3-Casp9 nucleotide sequence
  source 1..1554: mol_type = other DNA
atggcttctagaatcctctggcatgagatgtggcatgaaggcctggaagaggcatctcgtttgtactttggggaaaggaacgtgaaaggcatgtttgaggtgctggagcccttgcatgctatgatggaacggggcccccagactctgaaggaaacatcctttaatcaggcctatggtcgagatttaatggaggcccaagagtggtgcaggaagtacatgaaatcagggaatgtcaaggacctcctccaagcctgggacctctattatcatgtgttccgacgaatctcaaagctcgagtatagcggcggcggcagcctggagggcgtgcaggtggagaccatcagcccaggcgacggcagaaccttccccaagagaggccagacctgcgtggtgcactataccggcatgctggaggacggcaagaagttcgacagcagccgcgaccgcaataagcccttcaagttcatgctgggcaagcaggaggtgatcagaggctgggaggagggcgtggcccagatgagcgtgggccagagagccaagctgaccatcagccccgactacgcctatggcgccaccggccaccccggcatcatcccaccccacgccaccctggtgtttgatgtggagctgctgaagctggagtccggcggaggcgggtctggaggaggcggcagcggcggcggcgggtcaggcgtggatggcttcggcgacgtgggagccctggagagcctgagaggcaacgccgatctggcctacatcctgagcatggagccctgtggccactgcctgatcatcaacaacgtgaacttctgccgggagagcggcctgcggacccggaccggcagcaacatcgactgcgagaagctgaggaggcgcttctcctccctgcactttatggtggaggtgaaaggcgatctgactgccaagaaaatggtgctggccctgctggagctggcccagcaggaccacggagccctggattgctgtgtggtggtgatcctgtcccacggctgccaggccagccacctgcagttccccggagccgtgtacggcaccgacggctgtcccgtgtccgtggagaagatcgtgaacatcttcaacggcacctcctgcccctccctgggcggcaagcccaagctgttctttatccaggcctgtggcggcgagcagaaggaccacggctttgaggtggccagcacctcccccgaggacgagagcccaggcagcaaccccgagcccgacgccacccccttccaggagggcctgcgcaccttcgaccagctggacgccatcagcagcctgcccacccccagcgacatcttcgtgagctacagcacctttcccggcttcgtgagctggcgcgatcccaagtccggctcttggtatgtggagaccctggacgacatctttgagcagtgggctcatagcgaggacctgcagagcctgctgctgcgcgtggccaatgccgtgagcgtgaagggcatctacaagcagatgccaggctgcttcaacttcctgcggaagaagctgttcttcaagaccagcgcctcctga

SEQ ID NO: 13 - DNA, 1209 bp, synthetic construct
  misc_feature 1..1209: note = FKBP12-dCasp9 nucleotide sequence
  source 1..1209: mol_type = other DNA
atgctggagggcgtgcaggtggagaccatcagcccaggcgacggcagaaccttccccaagagaggccagacctgcgtggtgcactataccggcatgctggaggacggcaagaagttcgacagcagccgcgaccgcaataagcccttcaagttcatgctgggcaagcaggaggtgatcagaggctgggaggagggcgtggcccagatgagcgtgggccagagagccaagctgaccatcagccccgactacgcctatggcgccaccggccaccccggcatcatcccaccccacgccaccctggtgtttgatgtggagctgctgaagctggagtccggaggcggctccggcgtggatggcttcggcgacgtgggagccctggagagcctgagaggcaacgccgatctggcctacatcctgagcatggagccctgtggccactgcctgatcatcaacaacgtgaacttctgccgggagagcggcctgcggacccggaccggcagcaacatcgactgcgagaagctgaggaggcgcttctcctccctgcactttatggtggaggtgaaaggcgatctgactgccaagaaaatggtgctggccctgctggagctggcccagcaggaccacggagccctggattgctgtgtggtggtgatcctgtcccacggctgccaggccagccacctgcagttccccggagccgtgtacggcaccgacggctgtcccgtgtccgtggagaagatcgtgaacatcttcaacggcacctcctgcccctccctgggcggcaagcccaagctgttctttatccaggcctgtggcggcgagcagaaggaccacggctttgaggtggccagcacctcccccgaggacgagagcccaggcagcaaccccgagcccgacgccacccccttccaggagggcctgcgcaccttcgaccagctggacgccatcagcagcctgcccacccccagcgacatcttcgtgagctacagcacctttcccggcttcgtgagctggcgcgatcccaagtccggctcttggtatgtggagaccctggacgacatctttgagcagtgggctcatagcgaggacctgcagagcctgctgctgcgcgtggccaatgccgtgagcgtgaagggcatctacaagcagatgccaggctgcttcaacttcctgcggaagaagctgttcttcaagaccagcgcctcctga

SEQ ID NO: 14 - DNA, 1179 bp, synthetic construct
  misc_feature 1..1179: note = FRB-dCasp9 nucleotide sequence
  source 1..1179: mol_type = other DNA
atggcttctagaatcctctggcatgagatgtggcatgaaggcctggaagaggcatctcgtttgtactttggggaaaggaacgtgaaaggcatgtttgaggtgctggagcccttgcatgctatgatggaacggggcccccagactctgaaggaaacatcctttaatcaggcctatggtcgagatttaatggaggcccaagagtggtgcaggaagtacatgaaatcagggaatgtcaaggacctcctccaagcctgggacctctattatcatgtgttccgacgaatctcaaagctcgagtatagcggcggcggcagcggcgtggatggcttcggcgacgtgggagccctggagagcctgagaggcaacgccgatctggcctacatcctgagcatggagccctgtggccactgcctgatcatcaacaacgtgaacttctgccgggagagcggcctgcggacccggaccggcagcaacatcgactgcgagaagctgaggaggcgcttctcctccctgcactttatggtggaggtgaaaggcgatctgactgccaagaaaatggtgctggccctgctggagctggcccagcaggaccacggagccctggattgctgtgtggtggtgatcctgtcccacggctgccaggccagccacctgcagttccccggagccgtgtacggcaccgacggctgtcccgtgtccgtggagaagatcgtgaacatcttcaacggcacctcctgcccctccctgggcggcaagcccaagctgttctttatccaggcctgtggcggcgagcagaaggaccacggctttgaggtggccagcacctcccccgaggacgagagcccaggcagcaaccccgagcccgacgccacccccttccaggagggcctgcgcaccttcgaccagctggacgccatcagcagcctgcccacccccagcgacatcttcgtgagctacagcacctttcccggcttcgtgagctggcgcgatcccaagtccggctcttggtatgtggagaccctggacgacatctttgagcagtgggctcatagcgaggacctgcagagcctgctgctgcgcgtggccaatgccgtgagcgtgaagggcatctacaagcagatgccaggctgcttcaacttcctgcggaagaagctgttcttcaagaccagcgcctcctga

SEQ ID NO: 15 - DNA, 1956 bp, synthetic construct
  misc_feature 1..1956: note = FKBP12-Casp9-2A-FRB-FRBw nucleotide sequence
  source 1..1956: mol_type = other DNA
atgctggagggcgtgcaggtggagaccatcagcccaggcgacggcagaaccttccccaagagaggccagacctgcgtggtgcactataccggcatgctggaggacggcaagaagttcgacagcagccgcgaccgcaataagcccttcaagttcatgctgggcaagcaggaggtgatcagaggctgggaggagggcgtggcccagatgagcgtgggccagagagccaagctgaccatcagccccgactacgcctatggcgccaccggccaccccggcatcatcccaccccacgccaccctggtgtttgatgtggagctgctgaagctggagtccggaggcggctccggcgtggatggcttcggcgacgtgggagccctggagagcctgagaggcaacgccgatctggcctacatcctgagcatggagccctgtggccactgcctgatcatcaacaacgtgaacttctgccgggagagcggcctgcggacccggaccggcagcaacatcgactgcgagaagctgaggaggcgcttctcctccctgcactttatggtggaggtgaaaggcgatctgactgccaagaaaatggtgctggccctgctggagctggcccagcaggaccacggagccctggattgctgtgtggtggtgatcctgtcccacggctgccaggccagccacctgcagttccccggagccgtgtacggcaccgacggctgtcccgtgtccgtggagaagatcgtgaacatcttcaacggcacctcctgcccctccctgggcggcaagcccaagctgttctttatccaggcctgtggcggcgagcagaaggaccacggctttgaggtggccagcacctcccccgaggacgagagcccaggcagcaaccccgagcccgacgccacccccttccaggagggcctgcgcaccttcgaccagctggacgccatcagcagcctgcccacccccagcgacatcttcgtgagctacagcacctttcccggcttcgtgagctggcgcgatcccaagtccggctcttggtatgtggagaccctggacgacatctttgagcagtgggctcatagcgaggacctgcagagcctgctgctgcgcgtggccaatgccgtgagcgtgaagggcatctacaagcagatgccaggctgcttcaacttcctgcggaagaagctgttcttcaagaccagcgcctcccagtgcaccaattatgctttgcttaagctggcaggcgatgtggaatcaaacccgggtcctggggtacaggtggagaccatctctcctggcgacgggagaacatttcctaaaaggggccaaacatgcgtggttcactataccggtatgctggaggatggcaaaaaagtagactccagccgggatagaaacaaaccctttaagttcatgctgggtaagcaggaagttatacggggctgggaagagggagtagctcagatgtctgtgggccagagggccaagctgaccatctcaccggactacgcctacggcgctaccggccaccctggcattataccaccccatgcaactctcgtcttcgatgttgagttgctcaaactggaatcaggcggaggcgggtctggaggaggcggcagcatgctggagggcgtgcaggtggagaccatcagcccaggcgacggcagaaccttccccaagagaggccagacctgcgtggtgcactataccggcatgctggaggacggcaagaagttcgacagcagccgcgaccgcaataagcccttcaagttcatgctgggcaagcaggaggtgatcagaggctgggaggagggcgtggcccagatgagcgtgggccagagagccaagctgaccatcagccccgactacgcctatggcgccaccggccaccccggcatcatcccaccccacgccaccctggtgtttgatgtggagctgctgaagctggagtcctga

SEQ ID NO: 16 - protein, 20 aa, Foot-and-mouth disease virus
RAEGRGSLLTCGDVEENPGP

SEQ ID NO: 17 - protein, 20 aa, Foot-and-mouth disease virus
QCTNYALLKLAGDVESNPGP